European Patent Application EP 4 112 733 A1, published January 4, 2023. Title: Method for Synthesizing a Chiral Diamine Compound. Applicant: Asymchem Laboratories (Tianjin) Co., Ltd. The sequence listing filed with the application follows.

SEQUENCE LISTING (4 sequences)

SEQ ID NO: 1 - protein, 459 aa, Transaminase(Chromobacterium violaceum DSM30191)
  VARIANT (1)..(459): TA4-V1
MQKQRTCSQWRELDAAHHLHPFTDTASLNQAGARVMTRGEGVYLWDCEGNKIIDGMAGLWCVNVGYGRKDFAEAARRQMEELPFYNTFYKTTHPAVVELSSLLAEVTPAGFDRVFYTNSGSESVDTMIRMVRRYWDVQGKPEKKTLIGRWWGYHGSTIGGASLGGFKYMHEQGDLPIPGMAHIEQPWWYKHGKDMTPDEFGVVAARWLEEKILEIGADKVAAFVGEPIQGAGGVIVPPATYWPEIERICRKYDVLLVADEVICGFGRTGEWFGHQHFGFQPDLFTAAKGLSSGYLPIGAVFVGKRVAEGLIAGGDFNHGFTYSGHPVCAAVAHANVAALRDEGIVQRVKDDIGPYMQKRWRETFSRFEHVDDVRGVGMLLAFTLVKNKAKRELFPDFGEIGTLCRDIFFRNNLIMDSCGDHIVCAPPLVMTRAEVDEMLAVAERCLEEFEQTLKARGLA

SEQ ID NO: 2 - protein, 459 aa, Transaminase(Chromobacterium violaceum DSM30191)
  VARIANT (1)..(459): TA4-V2
MQKQRTCSQWRELDAAHHLHPFTDTASLNQAGARVMTRGEGVYLWDCEGNKIIDGMAGLWCVNVGYGRKDFAEAARRQMEELPFYNTFYKTTHPAVVELSSLLAEVTPAGFDRVFYTNSGSESVDTMIRMVRRYWDVQGKPEKKTLIGRWWGYHGSTIGGASLGGFKYMHEQGDLPIPGMAHIEQPWWYKHGKDMTPDEFGVVAARWLEEKILEIGADKVAAFVGEPIQGAGGVIVPPATYWPEIERICRKYDVLLVADEVICGFGRTGEWFGHQHFGFQPDLFTAAKGLSSGYLPIGAVFVGKRVAEGLIAGGDFNHGFTYSGHPVCAAVAHANVAALRDEGIVQRVKDDIGPYMQKRWRETFSRFEHVDDVRGVGMLLAFTLVKNKAKRELFPDFGEIGTLCRDIFFRNNLIMDSCGDHIVAAPPLVMTRAEVDEMLAVAERCLEEFEQTLKARGLA

SEQ ID NO: 3 - protein, 459 aa, Transaminase(Chromobacterium violaceum DSM30191)
  VARIANT (1)..(459): TA4-V3
MQKQRTCSQWRELDAAHHLHPFTDTASLNQAGARVMTRGEGVYLWDCEGNKIIDGMAGLWCVNVGYGRKDFAEAARRQMEELPFYNTFYKTTHPAVVELSSLLAEVTPAGFDRVFYTNSGSESVDTMIRMVRRYWDVQGKPEKKTLIGRWWGYHGSTIGGASLGGFKYMHEQGDLPIPGMAHIEQPWWYKHGKDMTPDEFGVVAARWLEEKILEIGADKVAAFVGEPIQGAGGVIVPPATYWPEIERICRKYDVLLVADEVICGFGRTGEWFGHQHFGFQPDLFTAAKGLSSGYLPIGAVFVGKRVAEGLIAGGDFNHGFTYSGHPVCAAVAHANVAALRDEGIVQRVKDDIGPYMQKRWRETFSRFEHVDDVRGVGMLLAFTLVKNKAKRELFPDFGEIGTLCRDIFQRNNLIMDSCGDHIVSAPPLVMTRAEVDEMLAVAERCLEEFEQTLKARGLA

SEQ ID NO: 4 - protein, 459 aa, Transaminase(Chromobacterium violaceum DSM30191)
  VARIANT (1)..(459): TA4-V4
MQKQRTCSQWRELDAAHHLHPFTDTASLNQAGARVMTRGEGVYLWDCEGNKIIDGMAGLWCVNVGYGRKDFAEAARRQMEELPFYNTFYKTTHPAVVELSSLLAEVTPAGFDRVFYTNSGSESVDTMIRMVRRYWDVQGKPEKKTLIGRWWGYHGSTIGGASLGGFKYMHEQGDLPIPGMAHIEQPWWYKHGKDMTPDEFGVVAARWLEEKILEIGADKVAAFVGEPIQGAGGVIVPPATYWPEIERICRKYDVLLVADEVICGFGRTGEWFGHQHFGFQPDLFTAAKGLSSGYLPIGAVFVGKRVAEGLIAGGDFNHGFTYSGHPVCAAVAHANVAALRDEGIVQRVKDDIGPYMQKRWRETFSRFEHVDDVRGVGMLLAFTLVKNKAKRELFPDFGEIGTLCRDIFHRNNLIMDSCGDHIVSAPPLVMTRAEVDEMLAVAERCLEEFEQTLKARGLA